European Patent Specification EP 4 050 104 B1, published October 23, 2024. Title: Novel DNA polymerase III subunits gamma and tau variant and a method for producing L-lysine using the same. Applicant: CJ CheilJedang Corporation. The sequence listing filed with the application follows.

SEQUENCE LISTING (11 sequences)

SEQ ID NO: 1 - protein, 775 aa, Artificial Sequence
  (P43L)_DNA polymerase III subunits gamma and tau
MALYSKYRPASFGELVGQSQVTDPLSAALDSGRINHAYLFSGLRGCGKTSSARILARSLNCVEGPTSTPCGVCNSCVALAPGGPGTLDVTELDAASNNGVDDMRELRERANYAPAESRYRVFIIDEAHMISTQGFNALLKIVEEPPAHLIFIFATTEPDKMIGTIRSRTHNYPFRLLTPGDMRKVLKNAVDGEGVHVDDSVYPLVIRAGGGSPRDSLSILDQLIAGSGPEGLTYERALPLLGVTSFTLIDDSIHALASKDNASMFTTIDNVIEEGLEPRRFTIDLLDRLRDLMVLQAVPEALNLGLVDAPTDRADALIEQSTLFKGNELANLASMVNSGLDDMRGATSPRLLLEILCARLLLASNTVAGPAVSSSTDAAPAATPGGLTGIAAARAKAREYGQKKAAPAPAPTPAPEPVREQSLAPTPEPTPAAEPTSQPAPEPEPAREPVVEVREASVEKQPASSDPLETIRSRWSELRNIVEKQSVRTSIMLTEARVLGLRGDTLVLGHSTGALAARLNAADHNGILVKVLAEETGLQLKVECIVGTNPAEAGFTAQPAVQKSTWNPNYDSKPATPSAPAQPQTPKQESVPTEPEEPESSAETSGWGQPVKIGGPAPEAQTPTPPPAPVVPATPAAPAAGAAKPAWKERVEQAAANAAQQRQHRQGSSEPFERGVPLPPEPDLPPDPYGYPADEGFPERNQGFQQQPAPPVEQPAPEPATEPVPAVAPEPEVSQLSEEEQLIREADEEPGEMDRRDAKTIAMELLAQELGAKPL

SEQ ID NO: 2 - DNA, 2328 bp, Artificial Sequence
  (P43L)_dnaZX
gtggctttgtatagcaagtatcgaccggcaagttttggtgaactagttgggcagtcgcaagtgactgaccctctgtccgcagctttggatagcgggcgcatcaaccatgcgtaccttttttcgggtctgcgtggttgtggcaagacgtcgtcggcacgcatccttgcccggtccctcaactgcgtggaaggcccaacttccacgccgtgtggggtgtgtaattcttgcgtagcgctggccccgggtggccctggaacccttgatgtaacagagctcgacgccgcgagtaacaatggtgtcgatgacatgcgtgaactgcgcgaacgcgcgaactacgccccggcggaatctcgctaccgcgtgttcatcattgacgaagcccacatgatcagtacccaaggcttcaacgccttgctgaaaatcgttgaagagccaccagcgcacctgattttcatcttcgccaccaccgagccggacaaaatgatcggtacgatccgttcccgcacgcacaattacccattccgcctgctcaccccaggggatatgcgcaaagtgctgaaaaatgcggtcgatggcgaaggcgtccacgtcgacgattccgtttacccactggtcatccgcgccggcggcggcagcccccgcgacagcctctccatcctcgaccagctcatcgccggctcgggcccggagggcttgacatatgagcgcgccttgccgctgctcggtgtcacaagcttcacgcttatcgacgattcgatccatgcccttgcatctaaagacaacgcaagcatgttcaccacgatcgataacgtcatcgaagaaggcctcgaaccgcgacgcttcacgatcgacctcctcgaccgcctccgcgacttgatggtcctccaagccgtcccagaagcactaaacctcgggcttgtcgacgcccccaccgaccgcgccgacgccctaatcgaacaatccaccctgttcaaaggcaacgagctcgccaacctagcctccatggtgaactccggactcgacgacatgcgtggtgccacctcaccgcgcctccttctggaaatcctctgcgcccgactgctcctggcaagcaataccgtggcaggtccagcggtcagtagttcgactgacgctgcgcctgcagctactccgggtggtctcactggtattgctgctgcccgcgcgaaagcacgggagtatggacagaagaaggcagctccagctcctgcaccaactcctgcgcccgagccagtgcgcgaacagtctcttgcaccaacgcctgaaccaacgccagcggctgaacctacatctcagcccgcgccggaaccggaacccgccagggaaccagtggtggaagtgcgggaggcgagcgtcgaaaagcagcctgcaagcagtgatcccctcgaaaccattcgaagccgctggtcagagctgcgcaacatcgtggaaaaacaaagtgtgcgcacctcaatcatgctgaccgaagcgcgagttttgggactgcgaggcgataccctcgtgctcggtcacagcaccggggcgttggctgcgcgtttgaacgctgctgatcacaacggaattttggtcaaggtgttggctgaggaaactggtctgcagctcaaggtcgaatgcattgtgggcacgaacccagccgaagctggatttaccgcccagcctgctgtgcaaaagagcacgtggaaccccaactacgactccaaaccagccactccaagtgcgcctgcgcagcctcagacgcctaagcaagaatccgtgcccaccgagccagaggagcctgagagttcggctgaaacttcgggatgggggcaaccggtaaaaatcggtgggccagcacctgaggcacagactccaacgcctccgcctgctccggtggttccggctactcctgctgctccggctgcgggtgctgcgaaaccagcgtggaaggaacgcgtcgaacaagccgcggcaaatgcagcgcaacaacgtcagcatcgccagggcagctccgagcccttcgagcggggtgttccgctgccaccagaacctgacctgccaccggacccctatggatacccagctgacgagggtttccccgaacgaaaccaagggttccagcaacagccagcgcctcccgttgagcaaccagctcctgagcctgcgacggagccagttccagcagttgcgcctgagccggaggtcagccagctatctgaagaagagcagctgatccgcgaagcagacgaagagccaggtgaaatggatcgtcgtgatgcgaaaaccatcgcgatggaactgcttgctcaggaactcggcgcgaaacctttgtaa

SEQ ID NO: 3 - protein, 775 aa, Artificial Sequence
  (WT)_DNA polymerase III subunits gamma and tau
MALYSKYRPASFGELVGQSQVTDPLSAALDSGRINHAYLFSGPRGCGKTSSARILARSLNCVEGPTSTPCGVCNSCVALAPGGPGTLDVTELDAASNNGVDDMRELRERANYAPAESRYRVFIIDEAHMISTQGFNALLKIVEEPPAHLIFIFATTEPDKMIGTIRSRTHNYPFRLLTPGDMRKVLKNAVDGEGVHVDDSVYPLVIRAGGGSPRDSLSILDQLIAGSGPEGLTYERALPLLGVTSFTLIDDSIHALASKDNASMFTTIDNVIEEGLEPRRFTIDLLDRLRDLMVLQAVPEALNLGLVDAPTDRADALIEQSTLFKGNELANLASMVNSGLDDMRGATSPRLLLEILCARLLLASNTVAGPAVSSSTDAAPAATPGGLTGIAAARAKAREYGQKKAAPAPAPTPAPEPVREQSLAPTPEPTPAAEPTSQPAPEPEPAREPVVEVREASVEKQPASSDPLETIRSRWSELRNIVEKQSVRTSIMLTEARVLGLRGDTLVLGHSTGALAARLNAADHNGILVKVLAEETGLQLKVECIVGTNPAEAGFTAQPAVQKSTWNPNYDSKPATPSAPAQPQTPKQESVPTEPEEPESSAETSGWGQPVKIGGPAPEAQTPTPPPAPVVPATPAAPAAGAAKPAWKERVEQAAANAAQQRQHRQGSSEPFERGVPLPPEPDLPPDPYGYPADEGFPERNQGFQQQPAPPVEQPAPEPATEPVPAVAPEPEVSQLSEEEQLIREADEEPGEMDRRDAKTIAMELLAQELGAKPL

SEQ ID NO: 4 - DNA, 2328 bp, Artificial Sequence
  (WT)_dnaZX
gtggctttgtatagcaagtatcgaccggcaagttttggtgaactagttgggcagtcgcaagtgactgaccctctgtccgcagctttggatagcgggcgcatcaaccatgcgtaccttttttcgggtccgcgtggttgtggcaagacgtcgtcggcacgcatccttgcccggtccctcaactgcgtggaaggcccaacttccacgccgtgtggggtgtgtaattcttgcgtagcgctggccccgggtggccctggaacccttgatgtaacagagctcgacgccgcgagtaacaatggtgtcgatgacatgcgtgaactgcgcgaacgcgcgaactacgccccggcggaatctcgctaccgcgtgttcatcattgacgaagcccacatgatcagtacccaaggcttcaacgccttgctgaaaatcgttgaagagccaccagcgcacctgattttcatcttcgccaccaccgagccggacaaaatgatcggtacgatccgttcccgcacgcacaattacccattccgcctgctcaccccaggggatatgcgcaaagtgctgaaaaatgcggtcgatggcgaaggcgtccacgtcgacgattccgtttacccactggtcatccgcgccggcggcggcagcccccgcgacagcctctccatcctcgaccagctcatcgccggctcgggcccggagggcttgacatatgagcgcgccttgccgctgctcggtgtcacaagcttcacgcttatcgacgattcgatccatgcccttgcatctaaagacaacgcaagcatgttcaccacgatcgataacgtcatcgaagaaggcctcgaaccgcgacgcttcacgatcgacctcctcgaccgcctccgcgacttgatggtcctccaagccgtcccagaagcactaaacctcgggcttgtcgacgcccccaccgaccgcgccgacgccctaatcgaacaatccaccctgttcaaaggcaacgagctcgccaacctagcctccatggtgaactccggactcgacgacatgcgtggtgccacctcaccgcgcctccttctggaaatcctctgcgcccgactgctcctggcaagcaataccgtggcaggtccagcggtcagtagttcgactgacgctgcgcctgcagctactccgggtggtctcactggtattgctgctgcccgcgcgaaagcacgggagtatggacagaagaaggcagctccagctcctgcaccaactcctgcgcccgagccagtgcgcgaacagtctcttgcaccaacgcctgaaccaacgccagcggctgaacctacatctcagcccgcgccggaaccggaacccgccagggaaccagtggtggaagtgcgggaggcgagcgtcgaaaagcagcctgcaagcagtgatcccctcgaaaccattcgaagccgctggtcagagctgcgcaacatcgtggaaaaacaaagtgtgcgcacctcaatcatgctgaccgaagcgcgagttttgggactgcgaggcgataccctcgtgctcggtcacagcaccggggcgttggctgcgcgtttgaacgctgctgatcacaacggaattttggtcaaggtgttggctgaggaaactggtctgcagctcaaggtcgaatgcattgtgggcacgaacccagccgaagctggatttaccgcccagcctgctgtgcaaaagagcacgtggaaccccaactacgactccaaaccagccactccaagtgcgcctgcgcagcctcagacgcctaagcaagaatccgtgcccaccgagccagaggagcctgagagttcggctgaaacttcgggatgggggcaaccggtaaaaatcggtgggccagcacctgaggcacagactccaacgcctccgcctgctccggtggttccggctactcctgctgctccggctgcgggtgctgcgaaaccagcgtggaaggaacgcgtcgaacaagccgcggcaaatgcagcgcaacaacgtcagcatcgccagggcagctccgagcccttcgagcggggtgttccgctgccaccagaacctgacctgccaccggacccctatggatacccagctgacgagggtttccccgaacgaaaccaagggttccagcaacagccagcgcctcccgttgagcaaccagctcctgagcctgcgacggagccagttccagcagttgcgcctgagccggaggtcagccagctatctgaagaagagcagctgatccgcgaagcagacgaagagccaggtgaaatggatcgtcgtgatgcgaaaaccatcgcgatggaactgcttgctcaggaactcggcgcgaaacctttgtaa

SEQ ID NO: 5 - DNA, 36 bp, Artificial Sequence
  dnaZX_1F
tcgagctcggtacccccaagagggtttttctgtggt

SEQ ID NO: 6 - DNA, 44 bp, Artificial Sequence
  dnaZX_2R
cgtcttgccacaaccacgcagacccgaaaaaaggtacgcatggt

SEQ ID NO: 7 - DNA, 44 bp, Artificial Sequence
  dnaZX_3F
accatgcgtaccttttttcgggtctgcgtggttgtggcaagacg

SEQ ID NO: 8 - DNA, 36 bp, Artificial Sequence
  dnaZX_4R
ctctagaggatccccgccgccgccggcgcggatgac

SEQ ID NO: 9 - DNA, 21 bp, Artificial Sequence
  dnaZX_5F
ccaagagggtttttctgtggt

SEQ ID NO: 10 - DNA, 21 bp, Artificial Sequence
  dnaZX_6R
gccgccgccggcgcggatgac

SEQ ID NO: 11 - DNA, 5803 bp, Artificial Sequence
  pDCM2_plasmid
gttcgcttgctgtccataaaaccgcccagtctagctatcgccatgtaagcccactgcaagctacctgctttctctttgcgcttgcgttttcccttgtccagatagcccagtagctgacattcatccggggtcagcaccgtttctgcggactggctttctacgtgttccgcttcctttagcagcccttgcgccctgagtgcttgcggcagcgtgaagctagcttttatcgccattcgccattcaggctgcgcaactgttgggaagggcgatcggtgcgggcctcttcgctattacgccagctggcgaaagggggatgtgctgcaaggcgattaagttgggtaacgccagggttttcccagtcacgacgttgtaaaacgacggccagtgaattcgagctcggtacccggggatcctctagagtcgacctgcaggcatgcaagcttggcgtaatcatggtcatagctgtttcctgtgtgaaattgttatccgctcacaattccacacaacatacgagccggaagcataaagtgtaaagcctggggtgcctaatgagtgagctaactcacattaattgcgttgcgctcactgcccgctttccagtcgggaaacctgtcgtgccagctgcattaatgaatcggccaacgcgcggggagaggcggtttgcgtattgggcgctcttccgcttcctcgctcactgactcgctgcgctcggtcgttcggctgcggcgagcggtatcagctcactcaaaggcggtaatacggttatccacagaatcaggggataacgcaggaaagaacatgtgagcaaaaggccagcaaaaggccaggaaccgtaaaaaggccgcgttgctggcgtttttccataggctccgcccccctgacgagcatcacaaaaatcgacgctcaagtcagaggtggcgaaacccgacaggactataaagataccaggcgtttccccctggaagctccctcgtgcgctctcctgttccgaccctgccgcttaccggatacctgtccgcctttctcccttcgggaagcgtggcgctttctcaatgctcacgctgtaggtatctcagttcggtgtaggtcgttcgctccaagctgggctgtgtgcacgaaccccccgttcagcccgaccgctgcgccttatccggtaactatcgtcttgagtccaacccggtaagacacgacttatcgccactggcagcagccactggtaacaggattagcagagcgaggtatgtaggcggtgctacagagttcttgaagtggtggcctaactacggctacactagaaggacagtatttggtatctgcgctctgctgaagccagttaccttcggaaaaagagttggtagctcttgatccggcaaacaaaccaccgctggtagcggtggtttttttgtttgcaagcagcagattacgcgcagaaaaaaaggatctcaagaagatcctttgatcttttctacggggtctgacgctcagtggaacgaaaactcacgttaagggattttggtcatgagattatcaaaaaggatcttcacctagatccttttggggtgggcgaagaactccagcatgagatccccgcgctggaggatcatccagccctgatagaaacagaagccactggagcacctcaaaaacaccatcatacactaaatcagtaagttggcagcatcacccgacgcactttgcgccgaataaatacctgtgacggaagatcacttcgcagaataaataaatcctggtgtccctgttgataccgggaagccctgggccaacttttggcgaaaatgagacgttgatcggcacgtaagaggttccaactttcaccataatgaaataagatcactaccgggcgtattttttgagttatcgagattttcaggagctgatagaaacagaagccactggagcacctcaaaaacaccatcatacactaaatcagtaagttggcagcatcacccgacgcactttgcgccgaataaatacctgtgacggaagatcacttcgcagaataaataaatcctggtgtccctgttgataccgggaagccctgggccaacttttggcgaaaatgagacgttgatcggcacgtaagaggttccaactttcaccataatgaaataagatcactaccgggcgtattttttgagttatcgagattttcaggagctctttggcatcgtctctcgcctgtcccctcagttcagtaatttcctgcatttgcctgtttccagtcggtagatattccacaaaacagcagggaagcagcgcttttccgctgcataaccctgcttcggggtcattatagcgattttttcggtatatccatcctttttcgcacgatatacaggattttgccaaagggttcgtgtagactttccttggtgtatccaacggcgtcagccgggcaggataggtgaagtaggcccacccgcgagcgggtgttccttcttcactgtcccttattcgcacctggcggtgctcaacgggaatcctgctctgcgaggctggccggctaccgccggcgtaacagatgagggcaagcggatggctgatgaaaccaagccaaccaggaagggcagcccacctatcaaggtgtactgccttccagacgaacgaagagcgattgaggaaaaggcggcggcggccggcatgagcctgtcggcctacctgctggccgtcggccagggctacaaaatcacgggcgtcgtggactatgagcacgtccgcgagggcgtcccggaaaacgattccgaagcccaacctttcatagaaggcggcggtggaatcgaaatctcgtgatggcaggttgggcgtcgcttggtcggtcatttcgaaaaaggttaggaatacggttagccatttgcctgcttttatatagttcantatgggattcacctttatgttgataagaaataaaagaaaatgccaataggatatcggcattttcttttgcgtttttatttgttaactgttaattgtccttgttcaaggatgctgtctttgacaacagatgttttcttgcctttgatgttcagcaggaagctcggcgcaaacgttgattgtttgtctgcgtagaatcctctgtttgtcatatagcttgtaatcacgacattgtttcctttcgcttgaggtacagcgaagtgtgagtaagtaaaggttacatcgttaggcggatcaagatccatttttaacacaaggccagttttgttcagcggcttgtatgggccagttaaagaattagaaacataaccaagcatgtaaatatcgttagacgtaatgccgtcaatcgtcatttttgatccgcgggagtcagtgaacaggtaccatttgccgttcattttaaagacgttcgcgcgttcaatttcatctgttactgtgttagatgcaatcagcggtttcatcacttttttcagtgtgtaatcatcgtttagctcaatcataccgagagcgccgtttgctaactcagccgtgcgttttttatcgctttgcagaagtttttgactttcttgacggaagaatgatgtgcttttgccatagtatgctttgttaaataaagattcttcgccttggtagccatcttcagttccagtgtttgcttcaaatactaagtatttgtggcctttatcttctacgtagtgaggatctctcagcgtatggttgtcgcctgagctgtagttgccttcatcgatgaactgctgtacattttgatacgtttttccgtcaccgtcaaagattgatttataatcctctacaccgttgatgttcaaagagctgtctgatgctgatacgttaacttgtgcagttgtcagtgtttgtttgccgtaatgtttaccggagaaatcagtgtagaataaacggatttttccgtcagatgtaaatgtggctgaacctgaccattcttgtgtttggtcttttaggatagaatcatttgcatcgaatttgtcgctgtctttaaagacgcggccagcgtttttccagctgtcaatagaagtttcgccgactttttgatagaacatgtaaatcgatgtgtcatccgcatttttaggatctccggctaatgcaaagacgatgtggtagccgtgatagtttgcgacagtgccgtcagcgttttgtaatggccagctgtcccaaacgtccaggccttttgcagaagagatatttttaattgtggacgaatcaaattcagaaacttgatatttttcatttttttgctgttcagggatttgcagcatatcatggcgtgtaatatgggaaatgccgtatgtttccttatatggcttttggttcgtttctttcgcaaacgcttgagttgcgcctcctgccagcagtgcggtagtaaaggttaatactgttgcttgttttgcaaactttttgatgttcatcgttcatgtctccttttttatgtactgtgttagcggtctgcttcttccagccctcctgtttgaagatggcaagttagttacgcacaataaaaaaagacctaaaatatgtaaggggtgacgccaaagtatacactttgccctttacacattttaggtcttgcctgctttatcagtaacaaacccgcgcgatttacttttcgacctcattctattagactctcgtttggattgcaactggtctattttcctcttttgtttgatagaaaatcataaaaggatttgcagactacgggcctaaagaactaaaaaatctatctgtttcttttcattctctgtattttttatagtttctgttgcatgggcataaagttgcctttttaatcacaattcagaaaatatcataatatctcatttcactaaataatagtgaacggcaggtatatgtgatgggttaaaaaggatcaccccagagtcccgctcagaagaactcgtcaagaaggcgatagaaggcgatgcgctgcgaatcgggagcggcgataccgtaaagcacgaggaagcggtcagcccattcgccgccaagctcttcagcaatatcacgggtagccaacgctatgtcctgatagcggtccgccacacccagccggccacagtcgatgaatccagaaaagcggccattttccaccatgatattcggcaagcaggcatcgccatgggtcacgacgagatcctcgccgtcgggcatccgcgccttgagcctggcgaacagttcggctggcgcgagcccctgatgctcttcgtccagatcatcctgatcgacaagaccggcttccatccgagtacgtgctcgctcgatgcgatgtttcgcttggtggtcgaatgggcaggtagccggatcaagcgtatgcagccgccgcattgcatcagccatgatggatactttctcggcaggagcaaggtgagatgacaggagatcctgccccggcacttcgcccaatagcagccagtcccttcccgcttcagtgacaacgtcgagacagctgcgcaaggaacgcccgtcgtggccagccacgatagccgcgctgcctcgtcttggagttcattcagggcaccggacaggtcggtcttgacaaaaagaaccgggcgcccctgcgctgacagccggaacacggcggcatcagagcagccgattgtctgttgtgcccagtcatagccgaatagcctctccacccaagcggccggagaacctgcgtgcaatccatcttgttcaatcatgcgaaacgatcctcatcctgtctcttgatcagatcttgatcccctgcgccatcagatccttggcggcaagaaagccatccagtttactttgcagggcttcccaaccttaccagagggcgccccagctggcaattccg